European Patent Specification EP 3 845 903 B1, published May 6, 2026. Title: Immunochromatography kit and method for detection of Mycobacterium tuberculosis. Applicant: FUJIFILM Corporation. The sequence listing filed with the application follows.

SEQUENCE LISTING (18 sequences)

SEQ ID NO: 1 - protein, 6 aa, HOMO SAPIENS
RSIRSA

SEQ ID NO: 2 - protein, 3 aa, HOMO SAPIENS
GAS

SEQ ID NO: 3 - protein, 9 aa, HOMO SAPIENS
QQYDFWYTF

SEQ ID NO: 4 - protein, 8 aa, HOMO SAPIENS
GFNFEDFG

SEQ ID NO: 5 - protein, 8 aa, HOMO SAPIENS
ISWNGANI

SEQ ID NO: 6 - protein, 13 aa, HOMO SAPIENS
IDWYRDDYYKMDV

SEQ ID NO: 7 - DNA, 1356 bp, homo sapiens
caagtgcagctgttggagtctgggggaggtgtggtacggccgggggggtccctgagactctcctgtgcagcctctggattcaactttgaagattttggcatgagctgggtccgccaagctccagggaaggggctggagtgggtctctagtattagttggaatggtgctaatataggctatgtagactctgtgaagggccgattcaccatctccagagacaacgccaagaactccctatatctgcaaatgaacagtctgagagccgaggacacggccttatattactgtgcgatagactggtacagagacgactactacaagatggacgtctggggcaaagggaccacggtcaccgtctcctcagcctcgaccaagggcccatcggtcttcccgctagcgccctcctccaagagcacctctgggggcacagcggccctgggctgcctggtcaaggactacttccccgaacctgtgacggtctcgtggaactcaggcgccctgaccagcggcgtgcacaccttcccggctgtcctacagtcctcaggactctactccctcagcagcgtggtgaccgtgccctccagcagcttgggcacccagacctacatctgcaacgtgaatcacaagcccagcaacaccaaggtggacaagaaagttgagcccaaatcttgtgacaaaactcacacatgcccaccgtgcccagcacctgaactcctggggggaccgtcagtcttcctcttccccccaaaacccaaggacaccctcatgatctcccggacccctgaggtcacatgcgtggtggtggacgtgagccacgaagaccctgaggtcaagttcaactggtacgtggacggcgtggaggtgcataatgccaagacaaagccgcgggaggagcagtacaacagcacgtaccgtgtggtcagcgtcctcaccgtcctgcaccaggactggctgaatggcaaggagtacaagtgcaaggtctccaacaaagccctcccagcccccatcgagaaaaccatctccaaagccaaagggcagccccgagaaccacaggtgtacaccctgcccccatcccgggatgagctgaccaagaaccaggtcagcctgacctgcctggtcaaaggcttctatcccagcgacatcgccgtggagtgggagagcaatgggcagccggagaacaactacaagaccacgcctcccgtgctggactccgacggctccttcttcctctacagcaagctcaccgtggacaagagcaggtggcagcaggggaacgtcttctcatgctccgtgatgcatgaggctctgcacaaccactacacgcagaagagcctctccctgtctccgggtaaatga

SEQ ID NO: 8 - protein, 451 aa, HOMO SAPIENS
QVQLLESGGGVVRPGGSLRLSCAASGFNFEDFGMSWVRQAPGKGLEWVSSISWNGANIGYVDSVKGRFTISRDNAKNSLYLQMNSLRAEDTALYYCAIDWYRDDYYKMDVWGKGTTVTVSSASTKGPSVFPLAPSSKSTSGGTAALGCLVKDYFPEPVTVSWNSGALTSGVHTFPAVLQSSGLYSLSSVVTVPSSSLGTQTYICNVNHKPSNTKVDKKVEPKSCDKTHTCPPCPAPELLGGPSVFLFPPKPKDTLMISRTPEVTCVVVDVSHEDPEVKFNWYVDGVEVHNAKTKPREEQYNSTYRVVSVLTVLHQDWLNGKEYKCKVSNKALPAPIEKTISKAKGQPREPQVYTLPPSRDELTKNQVSLTCLVKGFYPSDIAVEWESNGQPENNYKTTPPVLDSDGSFFLYSKLTVDKSRWQQGNVFSCSVMHEALHNHYTQKSLSLSPGK

SEQ ID NO: 9 - DNA, 642 bp, HOMO SAPIENS
gaaatagtgatgacgcagtctccagccaccctgtctgtctctccaggggaaagagccaccctctcctgcagggccagtcggagtattcgcagcgccttagcctggtaccagcacaaacctggccaggctcccaggctcctcatctttggtgcatccaccagggccactggtatcccagccaggttcagtggcagtgggtctgggacagacttcactctcaccgtcagcagcatacggtctgaggattctgcagtttattactgtcagcagtatgatttctggtacacttttggccaggggaccaagctggagatcaaacgaactgtggctgcaccatctgtcttcatcttcccgccatctgatgagcagttgaaatctggaactgcctctgttgtgtgcctgctgaataacttctatcccagagaggccaaagtacagtggaaggtcgacaacgccctccaatcgggtaactcccaggagagtgtcacagagcaggacagcaaggacagcacctacagcctcagcagcaccctgacgctgagcaaagcagactacgagaaacacaaagtctacgcctgcgaagtcacccatcagggcctgagctcgcccgtcacaaagagcttcaacaggggagagtgttag

SEQ ID NO: 10 - protein, 213 aa, HOMO SAPIENS
EIVMTQSPATLSVSPGERATLSCRASRSIRSALAWYQHKPGQAPRLLIFGASTRATGIPARFSGSGSGTDFTLTVSSIRSEDSAVYYCQQYDFWYTFGQGTKLEIKRTVAAPSVFIFPPSDEQLKSGTASVVCLLNNFYPREAKVQWKVDNALQSGNSQESVTEQDSKDSTYSLSSTLTLSKADYEKHKVYACEVTHQGLSSPVTKSFNRGEC

SEQ ID NO: 11 - protein, 5 aa, Leporidae
TYYMT

SEQ ID NO: 12 - protein, 16 aa, Leporidae
TIDSYGNRYYASWAKG

SEQ ID NO: 13 - protein, 10 aa, Leporidae
DDLGWNNDNI

SEQ ID NO: 14 - protein, 13 aa, Leporidae
QASESVYGNNQLA

SEQ ID NO: 15 - protein, 7 aa, Leporidae
KASTLAS

SEQ ID NO: 16 - protein, 13 aa, Leporidae
CGGYKGSTTDGAA

SEQ ID NO: 17 - protein, 119 aa, Leporidae
AQSVKESGGRLVTPGGSLTLTCTVSGIDLTTYYMTWIRQAPGKGLEWIGTIDSYGNRYYASWAKGQFTISKTSSTTVDLKMTGLTASDTATYFCTRDDLGWNNDNIWGPGTLVTVSSSS

SEQ ID NO: 18 - protein, 112 aa, Leporidae
ELVMTQTPSSKSVPVGDTVTINCQASESVYGNNQLAWYQQKPGQPPKLLIYKASTLASGVPSRFKGSGYGTQFTLTISDVVCDDAATYYCGGYKGSTTDGAAFGGGTEVVVK